European Patent Specification EP 3 930 760 B1, published January 10, 2024. Title: CELL MEMBRANE PENETRATING CONJUGATES. Applicant: CyCa OncoSolutions Limited. The sequence listing filed with the application follows.

SEQUENCE LISTING (29 sequences)

SEQ ID NO: 1 - protein, 200 aa, Artificial Sequence
  Amino acid sequence of AlbG protein
MPAKTLESKDYCGESFVSEDRSGQSLESIRFEDCTFRQCNFTEAELNRCKFRECEFVDCNLSLISIPQTSFMEVRFVDCKMLGVNWTSAQWPSVKMEGALSFERCILNDSLFYGLYLAGVKMVECRIHDANFTEADCEDADFTQSDLKGSTFHNTKLTGASFIDAVNYHIDIFHNDIKRARFSLPEAASLLNSLDIELSD

SEQ ID NO: 2 - protein, 214 aa, Artificial Sequence
  Amino acid sequence of EfsQNR protein
GSHMKITYPLPPNLPEQLPLLTNCQLEDEAILENHLYQQIDLPNQEVRNLVFRDAVFDHLSLANGQFASFDCSNVRFEACDFSNVEWLSGSFHRVTFLRCNLTGTNFADSYLKDCLFEDCKADYASFRFANFNLVHFNQTRLVESEFFEVTWKKLLLEACDLTESNWLNTSLKGLDFSQNTFERLTFSPNYLSGLKVTPEQAIYLASALGLVIT

SEQ ID NO: 3 - protein, 84 aa, Tenebrio molitor
  Amino acid sequence of anti-freeze protein from Tenebrio molitor
QCTGGADCTSCTGACTGCGNCPNAVTCTNSQHCVKANTCTGSTDCNTAQTCTNSKDCFEANTCTDSTNCYKATACTNSSGCPGH

SEQ ID NO: 4 - protein, 143 aa, Rhagium inquisitor
  Acid sequence of anti-freeze protein from Rhagium inquisitor
GYSCRAVGVDGRAVTDIQGTCHAKATGAGAMASGTSEPGSTSTATATGRGATARSTSTGRGTATTTATGTASATSNAIGQGTATTTATGSAGGRATGSATTSSSASQPTQTQTITGPGFQTAKSFARNTATTTVTASHHHHHH

SEQ ID NO: 5 - protein, 90 aa, Choristoneura fumiferana
  Amino acid sequence of anti-freeze protein from Spruce Budworm
DGSCTNTNSQLSANSKCEKSTLTNCYVDKSEVYGTTCTGSRFDGVTITTSTSTGSRISGPGCKISTCIITGGVPAPSAACKISGCTFSAN

SEQ ID NO: 6 - protein, 217 aa, Artificial Sequence
  Amino acid sequence of QNRB1 protein
GSHMALALVGEKIDRNRFTGEKIENSTFFNCDFSGADLSGTEFIGCQFYDRESQKGCNFSRAMLKDAIFKSCDLSMADFRNSSALGIEIRHCRAQGADFRGASFMNMITTRTWFCSAYITNTNLSYANFSKVVLEKCELWENRWIGAQVLGATFSGSDLSGGEFSTFDWRAANFTHCDLTNSELGDLDIRGVDLQGVKLDNYQASLLMERLGIAVIG

SEQ ID NO: 7 - protein, 262 aa, Artificial Sequence
  Amino acid sequence of UDP-N-acetylglucosamine acyltransferase protein
MIDKSAFVHPTAIVEEGASIGANAHIGPFCIVGPHVEIGEGTVLKSHVVVNGHTKIGRDNEIYQFASIGEVNQDLKYAGEPTRVEIGDRNRIRESVTIHRGTVQGGGLTKVGSDNLLMINAHIAHDCTVGNRCILANNATLAGHVSVDDFAIIGGMTAVHQFCIIGAHVMVGGCSGVAQDVPPYVIAQGNHATPFGVNIEGLKRRGFSREAITAIRNAYKLIYRSGKTLDEVKPEIAELAETYPEVKAFTDFFARSTRGLIR

SEQ ID NO: 8 - protein, 201 aa, Artificial Sequence
  Amino acid sequence of NP275 protein from Nostoc punctiforme
MGSSHHHHHHSSGLVPRGSHMDVEKLRQLYAAGERDFSIVDLRGAVLENINLSGAILHGAMLDEANLQQANLSRADLSGATLNGADLRGANLSKADLSDAILDNAILEGAILDEAVLNQANLKAANLEQAILSHANIREADLSEANLEAADLSGADLAIADLHQANLHQAALERANLTGANLEDANLEGTILEGGNNNLAT

SEQ ID NO: 9 - protein, 353 aa, Artificial Sequence
  Amino acid sequence of pectate lyase C protein
ATDTGGYAATAGGNVTGAVSKTATSMQDIVNIIDAARLDANGKKVKGGAYPLVITYTGNEDSLINAAAANICGQWSKDPRGVEIKEFTKGITIIGANGSSANFGIWIKKSSDVVVQNMRIGYLPGGAKDGDMIRVDDSPNVWVDHNELFAANHECDGTPDNDTTFESAVDIKGASNTVTVSYNYIHGVKKVGLDGSSSSDTGRNITYHHNYYNDVNARLPLQRGGLVHAYNNLYTNITGSGLNVRQNGQALIENNWFEKAINPVTSRYDGKNFGTWVLKGNNITKPADFSTYSITWTADTKPYVNADSWTSTGTFPTVAYNYSPVSAQCVKDKLPGYAGVGKNLATLTSTACK

SEQ ID NO: 10 - protein, 196 aa, Caldicellulosiruptor bescii
  Amino acid sequence of pectate lyase from Caldicellulosiruptor bescii
VGTNTGGVLVITDTIIVKSGQTYDGKGIKIIAQGMGDGSQSENQKPIFKLEKGANLKNVIIGAPGCDGIHCYGDNVVENVVWEDVGEDALTVKSEGVVEVIGGSAKEAADKVFQLNAPCTFKVKNFTATNIGKLVRQNGNTTFKVVIYLEDVTLNNVKSCVAKSDSPVSELWYHNLNVNNCKTLFEFPSQSQIHQY

SEQ ID NO: 11 - protein, 213 aa, Methanosarcina thermophila
  Amino acid sequence of carbonic anhydrase from Methanosarcina thermophila
QEITVDEFSNIRENPVTPWNPEPSAPVIDPTAYIDPQASVIGEVTIGANVMVSPMASIRSDEGMPIFVGDRSNVQDGVVLHALETINEEGEPIEDNIVEVDGKEYAVYIGNNVSLAHQSQVHGPAAVGDDTFIGMQAFVFKSKVGNNCVLEPRSAAIGVTIPDGRYIPAGMVVTSQAEADKLPEVTDDYAYSHTNEAVVYVNVHLAEGYKETS

SEQ ID NO: 12 - protein, 359 aa, Aspergillus niger
  Amino acid sequence of Pectin lyase A protein from Aspergillus niger
VGVSGSAEGFAKGVTGGGSATPVYPDTIDELVSYLGDDEARVIVLTKTFDFTDSEGTTTGTGCAPWGTASACQVAIDQDDWCENYEPDAPSVSVEYYNAGTLGITVTSNKSLIGEGSSGAIKGKGLRIVSGAENIIIQNIAVTDINPKYVWGGDAITLDDCDLVWIDHVTTARIGRQHYVLGTSADNRVSLTNNYIDGVSDYSATCDGYHYWAIYLDGDADLVTMKGNYIYHTSGRSPKVQDNTLLHAVNNYWYDISGHAFEIGEGGYVLAEGNVFQNVDTVLETYEGEAFTVPSSTAGEVCSTYLGRDCVINGFGSSGTFSEDSTSFLSDFEGKNIASASAYTSVASRVVANAGQGNL

SEQ ID NO: 13 - protein, 135 aa, Artificial Sequence
  Amino acid sequence of TtCuA protein
AYTLATHTAGVIPAGKLERVDPTTVRQEGPWADPAQAVVQTGPNQYTVYVLAFAFGYQPNPIEVPQGAEIVFKITSPDVIHGFHVEGTNINVEVLPGEVSTVRYTFKRPGEYRIICNQYCGLGHQNMFGTIVVKE

SEQ ID NO: 14 - protein, 9 aa, Artificial Sequence
  Signal sequence for targeting the nucleus of the cell
PAAKRVKCD

SEQ ID NO: 15 - protein, 13 aa, Artificial Sequence
  Signal sequence for targeting the endoplasmic reticulum of the cell
YPYDVPDYAKDEL

SEQ ID NO: 16 - protein, 25 aa, Artificial Sequence
  Signal sequence for targeting the mitochondria of the cell
MLSLRQSIRFFKPATRTLCSSRYLL

SEQ ID NO: 17 - protein, 28 aa, Artificial Sequence
  Signal sequence for targeting the P-cadherin-over expressing breast cancer cells
LSTAADMQGVVTDGMASGLDKDYLKPDD

SEQ ID NO: 18 - protein, 5 aa, Artificial Sequence
  Consensus sequence in a pentapeptide-repeat protein
  misc_feature (1)..(1): Ser or Thr or Ala or Val
  misc_feature (2)..(2): Asp or Asn
  misc_feature (3)..(3): Leu or Phe
  misc_feature (4)..(4): Ser or Thr or Arg
XXXXG

SEQ ID NO: 19 - DNA, 582 bp, Artificial Sequence
  Nucleic acid sequence of AlbG gene
atgccggcgaaaaccctggaaagcaaagattattgcggcgaaagctttgtgagcgaagatcgcagcggccagagcctggaaagcattcgctttgaagattgcacctttcgccagtgcaactttaccgaagcggaactgaaccgctgcaaatttcgcgaatgcgaatttgtggattgcaacctgagcctgattagcattccgcagaccagctttatggaagtgcgctttgtggattgcaaaatgctgggcgtgaactggaccagcgcgcaggcgggcgcgctgagctttgaacgctgcattctgaacgatagcctgttttatggcctgtatctggcgggcgtgaaaatggtggaatgccgcattcatgatgcgaactttaccgaagcggattgcgaagatgcggattttacccagagcgatctgaaaggcagcacctttcataacaccaaactgaccggcgcgagctttattgatgcggtgaactatcatattgatatttttcataacgatattaaacgcgcgcgctttagcctgccggaagcggcgagcctgctgaacagcctggatattgaactgagcgat

SEQ ID NO: 20 - DNA, 642 bp, Artificial Sequence
  nucleic acid sequence of EfsQNR gene
ggcagccatatgaaaattacctatccgctgccgccgaacctgccggaacagctgccgctgctgaccaactgccagctggaagatgaagcgattctggaaaaccatctgtatcagcagattgatctgccgaaccaggaagtgcgcaacctggtgtttcgcgatgcggtgtttgatcatctgagcctggcgaacggccagtttgcgagctttgattgcagcaacgtgcgctttgaagcgtgcgattttagcaacgtggaatggctgagcggcagctttcatcgcgtgacctttctgcgctgcaacctgaccggcaccaactttgcggatagctatctgaaagattgcctgtttgaagattgcaaagcggattatgcgagctttcgctttgcgaactttaacctggtgcattttaaccagacccgcctggtggaaagcgaattttttgaagtgacctggaaaaaactgctgctggaagcgtgcgatctgaccgaaagcaactggctgaacaccagcctgaaaggcctggattttagccagaacacctttgaacgcctgacctttagcccgaactatctgagcggcctgaaagtgaccccggaacaggcgatttatctggcgagcgcgctgggcctggtgattacc

SEQ ID NO: 21 - DNA, 405 bp, Artificial Sequence
  Nucleic acid sequence of TtCuA gene
gcgtataccctggcgacccataccgcgggcgtgattccggcgggcaaactggaacgcgtggatccgaccaccgtgcgccaggaaggcccgtgggcggatccggcgcaggcggtggtgcagaccggcccgaaccagtataccgtgtatgtgctggcgtttgcgtttggctatcagccgaacccgattgaagtgccgcagggcgcggaaattgtgtttaaaattaccagcccggatgtgattcatggctttcatgtggaaggcaccaacattaacgtggaagtgctgccgggcgaagtgagcaccgtgcgctatacctttaaacgcccgggcgaatatcgcattatttgcaaccagtattgcggcctgggccatcagaacatgtttggcaccattgtggtgaaagaa

SEQ ID NO: 22 - protein, 16 aa, Artificial Sequence
  Signal sequence for targeting actin in the cell
GDVQKKRWLFETKPLD

SEQ ID NO: 23 - protein, 18 aa, Artificial Sequence
  Signal sequence for targeting tubulin in the cell
VQSKCGSKDNIKHVPGGG

SEQ ID NO: 24 - protein, 90 aa, Artificial Sequence
  Amino acid sequence of a zinc finger protein
MERPYACPVESCDRRFSDSSNLTRHIRIHTGQKPFQCRICMRNFSRSDHLTTHIRTHTGEKPFACDICGRKFARSDERKRHTKIHLRQKD

SEQ ID NO: 25 - DNA, 740 bp, Artificial Sequence
  Nucleic acid sequence of mcherry gene
gtgagcaagggcgaggaggataacatggccatcatcaaggagttcatgcgcttcaaggtgcacatggagggctccgtgaacggccacgagttcgagatcgagggcgagggcgagggccgcccctacgagggcacccagaccgccaagctgaaggtgaccaagggtggccccctgcccttcgcctgggacatcctgtcccctcagttcatgtacggctccaaggcctacgtgaagcaccccgccgacatccccgactacttgaagctgtccttccccgagggcttcaagtgggagcgcgtgatgaacttcgaggacggcggcgtggtgaccgtgacccaggactcctccctccaggacggcgagttcatctacaaggtgaagctgcgcggcaccaacttcccctccgacggccccgtaatgcagaagaagaccatgggctgggaggcctcctccgagcggatgtaccccgaggacggcgccctgaagggcgagatcaagcagaggctgaagctgaaggacggcggccactacgacgctgaggtcaagaccacctacaaggccaagaagcccgtgcagctgcccggcgcctacaacgtcaacatcaagttggacatcacctcccacaacgaggactacaccatcgtggaacagtacgaacgcgccgagggccgccactccaccggcggcatggacgagctgtacaagtagtaatctagagggccctattctatagtgtcacc

SEQ ID NO: 26 - DNA, 30 bp, Artificial Sequence
  Nucleic acid sequence of a PCR primer AlbG gene
atcccgctcatatgccggccaagacccttg

SEQ ID NO: 27 - DNA, 35 bp, Artificial Sequence
  Nucleic acid sequence of a PCR primer AlbG gene
atcccgctctcgagtcaatcggacagctcgatatc

SEQ ID NO: 28 - DNA, 35 bp, Artificial Sequence
  Nucleic acid sequence of a PCR primer EfsQNR gene
atcccgctcatatgaaaataacttatcccttgcca

SEQ ID NO: 29 - DNA, 36 bp, Artificial Sequence
  Nucleic acid sequence of a PCR primer EfsQNR gene
atcccgctctcgagttaggtaatcaccaaaccaagt